European Patent Application EP 4 249 595 A1, published September 27, 2023. Title: Variant of D-allulose 3-epimerase with excellent heat stability, manufacturing method thereof and manufacturing method of D-alluose using the same. Applicant: DAESANG CORPORATION. The sequence listing filed with the application follows.

SEQUENCE LISTING (12 sequences)

SEQ ID NO: 1 - protein, 294 aa, Unknown
  Wild type D-allulose 3-epimerase derived from Flavonifractor plautii
MNPIGMHYGFWSHNWDEIAYIPLMEKLAWLGFDICEVASAEWGYYDDARLRELKACADHNGLGITYSIGLEAKYDLASDDPAVRENGIRHVTRILESMPKVGAAILNGVSYAGWQALPDHGITLDEKRRKEELALESMSRLMKVAEDCGVLYCCEVVNRFEQYLLNTAKEGVEFVKRLGSPNARVLLDTFHMNIEEDSMVDAILEAGPWLGHFHVGENNRRPAGSTNRLPWKDMAAALKQVNYQGAIVMEPFVLMGGTIPYDIKVWRDLSGGAGEAGLDEMAGRACRFLKELTA

SEQ ID NO: 2 - DNA, 885 bp, Unknown
  Polynucleotide coding wild type D-allulose 3-epimerase derived from Flavonifractor plautii
atgaacccgattggaatgcactacggcttctggagccacaactgggacgagattgcatacatacccctgatggagaagctggcctggctgggctttgacatctgcgaggtggcctccgccgagtggggctattacgacgacgccaggctgcgggagctgaaggcctgcgccgatcacaacggcctgggcatcacctattccatcggcctggaggccaaatacgacctggccagcgacgatccggcggtgcgggagaacggcatccgccatgtcacccgcatcctggagagcatgcccaaggtgggggcggccatcctcaacggcgtgtcctacgccgggtggcaggccctgcccgaccacggaatcaccctggacgagaagcgccgcaaggaggagcttgccctggagtccatgtcccggctcatgaaggtggcggaggactgcggcgtgctctactgctgcgaggtggtcaaccgcttcgagcagtacctgctcaacaccgccaaagagggcgtggagtttgtcaagcgcctgggcagtcccaacgcccgggtgctgctggataccttccacatgaacatcgaggaggacagcatggtggacgccattctggaggcgggcccctggctggggcatttccacgtgggggagaacaaccgccgccccgccggctccaccaaccgcctgccctggaaggacatggccgccgccctcaagcaggtgaactaccagggggccattgtgatggagcccttcgtgctcatggggggtaccattccctatgatatcaaggtctggcgggatctcagcggcggggccggggaggccgggctggacgagatggcgggccgggcctgccggttcctcaaggagctgaccgcgtaa

SEQ ID NO: 3 - protein, 294 aa, Artificial Sequence
  D-allulose 3-epimerase variant W29K/G216S/M234I
MNPIGMHYGFWSHNWDEIAYIPLMEKLAKLGFDICEVASAEWGYYDDARLRELKACADHNGLGITYSIGLEAKYDLASDDPAVRENGIRHVTRILESMPKVGAAILNGVSYAGWQALPDHGITLDEKRRKEELALESMSRLMKVAEDCGVLYCCEVVNRFEQYLLNTAKEGVEFVKRLGSPNARVLLDTFHMNIEEDSMVDAILEAGPWLGHFHVSENNRRPAGSTNRLPWKDIAAALKQVNYQGAIVMEPFVLMGGTIPYDIKVWRDLSGGAGEAGLDEMAGRACRFLKELTA

SEQ ID NO: 4 - DNA, 885 bp, Artificial Sequence
  Polynucleotide coding D-allulose 3-epimerase variant W29K/G216S/M234
atgaacccgattggaatgcactacggcttctggagccacaactgggacgagattgcatacatacccctgatggagaagctggccaaactgggctttgacatctgcgaggtggcctccgccgagtggggctattacgacgacgccaggctgcgggagctgaaggcctgcgccgatcacaacggcctgggcatcacctattccatcggcctggaggccaaatacgacctggccagcgacgatccggcggtgcgggagaacggcatccgccatgtcacccgcatcctggagagcatgcccaaggtgggggcggccatcctcaacggcgtgtcctacgccgggtggcaggccctgcccgaccacggaatcaccctggacgagaagcgccgcaaggaggagcttgccctggagtccatgtcccggctcatgaaggtggcggaggactgcggcgtgctctactgctgcgaggtggtcaaccgcttcgagcagtacctgctcaacaccgccaaagagggcgtggagtttgtcaagcgcctgggcagtcccaacgcccgggtgctgctggataccttccacatgaacatcgaggaggacagcatggtggacgccattctggaggcgggcccctggctggggcatttccacgtgagcgagaacaaccgccgccccgccggctccaccaaccgcctgccctggaaggacattgccgccgccctcaagcaggtgaactaccagggggccattgtgatggagcccttcgtgctcatggggggtaccattccctatgatatcaaggtctggcgggatctcagcggcggggccggggaggccgggctggacgagatggcgggccgggcctgccggttcctcaaggagctgaccgcgtaa

SEQ ID NO: 5 - protein, 294 aa, Artificial Sequence
  D-allulose 3-epimerase variant W29K/A77S/G216S/M234I
MNPIGMHYGFWSHNWDEIAYIPLMEKLAKLGFDICEVASAEWGYYDDARLRELKACADHNGLGITYSIGLEAKYDLSSDDPAVRENGIRHVTRILESMPKVGAAILNGVSYAGWQALPDHGITLDEKRRKEELALESMSRLMKVAEDCGVLYCCEVVNRFEQYLLNTAKEGVEFVKRLGSPNARVLLDTFHMNIEEDSMVDAILEAGPWLGHFHVSENNRRPAGSTNRLPWKDIAAALKQVNYQGAIVMEPFVLMGGTIPYDIKVWRDLSGGAGEAGLDEMAGRACRFLKELTA

SEQ ID NO: 6 - protein, 294 aa, Artificial Sequence
  D-allulose 3-epimerase variant W29K/E173A/G216S/M234I
MNPIGMHYGFWSHNWDEIAYIPLMEKLAKLGFDICEVASAEWGYYDDARLRELKACADHNGLGITYSIGLEAKYDLASDDPAVRENGIRHVTRILESMPKVGAAILNGVSYAGWQALPDHGITLDEKRRKEELALESMSRLMKVAEDCGVLYCCEVVNRFEQYLLNTAKEGVAFVKRLGSPNARVLLDTFHMNIEEDSMVDAILEAGPWLGHFHVSENNRRPAGSTNRLPWKDIAAALKQVNYQGAIVMEPFVLMGGTIPYDIKVWRDLSGGAGEAGLDEMAGRACRFLKELTA

SEQ ID NO: 7 - protein, 294 aa, Artificial Sequence
  D-allulose 3-epimerase variant W29K/W209L/G216S/M234I
MNPIGMHYGFWSHNWDEIAYIPLMEKLAKLGFDICEVASAEWGYYDDARLRELKACADHNGLGITYSIGLEAKYDLASDDPAVRENGIRHVTRILESMPKVGAAILNGVSYAGWQALPDHGITLDEKRRKEELALESMSRLMKVAEDCGVLYCCEVVNRFEQYLLNTAKEGVEFVKRLGSPNARVLLDTFHMNIEEDSMVDAILEAGPLLGHFHVSENNRRPAGSTNRLPWKDIAAALKQVNYQGAIVMEPFVLMGGTIPYDIKVWRDLSGGAGEAGLDEMAGRACRFLKELTA

SEQ ID NO: 8 - protein, 294 aa, Artificial Sequence
  D-allulose 3-epimerase variant W29K/G216S/M234I/Q240D
MNPIGMHYGFWSHNWDEIAYIPLMEKLAKLGFDICEVASAEWGYYDDARLRELKACADHNGLGITYSIGLEAKYDLASDDPAVRENGIRHVTRILESMPKVGAAILNGVSYAGWQALPDHGITLDEKRRKEELALESMSRLMKVAEDCGVLYCCEVVNRFEQYLLNTAKEGVEFVKRLGSPNARVLLDTFHMNIEEDSMVDAILEAGPWLGHFHVSENNRRPAGSTNRLPWKDIAAALKDVNYQGAIVMEPFVLMGGTIPYDIKVWRDLSGGAGEAGLDEMAGRACRFLKELTA

SEQ ID NO: 9 - DNA, 885 bp, Artificial Sequence
  Polynucleotide coding D-allulose 3-epimerase variant W29K/A77S/G216S/M234I
atgaacccgattggaatgcactacggcttctggagccacaactgggacgagattgcatacatacccctgatggagaagctggccaaactgggctttgacatctgcgaggtggcctccgccgagtggggctattacgacgacgccaggctgcgggagctgaaggcctgcgccgatcacaacggcctgggcatcacctattccatcggcctggaggccaaatacgacctgagcagcgacgatccggcggtgcgggagaacggcatccgccatgtcacccgcatcctggagagcatgcccaaggtgggggcggccatcctcaacggcgtgtcctacgccgggtggcaggccctgcccgaccacggaatcaccctggacgagaagcgccgcaaggaggagcttgccctggagtccatgtcccggctcatgaaggtggcggaggactgcggcgtgctctactgctgcgaggtggtcaaccgcttcgagcagtacctgctcaacaccgccaaagagggcgtggagtttgtcaagcgcctgggcagtcccaacgcccgggtgctgctggataccttccacatgaacatcgaggaggacagcatggtggacgccattctggaggcgggcccctggctggggcatttccacgtgagcgagaacaaccgccgccccgccggctccaccaaccgcctgccctggaaggacattgccgccgccctcaagcaggtgaactaccagggggccattgtgatggagcccttcgtgctcatggggggtaccattccctatgatatcaaggtctggcgggatctcagcggcggggccggggaggccgggctggacgagatggcgggccgggcctgccggttcctcaaggagctgaccgcgtaa

SEQ ID NO: 10 - DNA, 885 bp, Artificial Sequence
  Polynucleotide coding D-allulose 3-epimerase variant W29K/E173A/G216S/M234I
atgaacccgattggaatgcactacggcttctggagccacaactgggacgagattgcatacatacccctgatggagaagctggccaaactgggctttgacatctgcgaggtggcctccgccgagtggggctattacgacgacgccaggctgcgggagctgaaggcctgcgccgatcacaacggcctgggcatcacctattccatcggcctggaggccaaatacgacctggccagcgacgatccggcggtgcgggagaacggcatccgccatgtcacccgcatcctggagagcatgcccaaggtgggggcggccatcctcaacggcgtgtcctacgccgggtggcaggccctgcccgaccacggaatcaccctggacgagaagcgccgcaaggaggagcttgccctggagtccatgtcccggctcatgaaggtggcggaggactgcggcgtgctctactgctgcgaggtggtcaaccgcttcgagcagtacctgctcaacaccgccaaagagggcgtggcgtttgtcaagcgcctgggcagtcccaacgcccgggtgctgctggataccttccacatgaacatcgaggaggacagcatggtggacgccattctggaggcgggcccctggctggggcatttccacgtgagcgagaacaaccgccgccccgccggctccaccaaccgcctgccctggaaggacattgccgccgccctcaagcaggtgaactaccagggggccattgtgatggagcccttcgtgctcatggggggtaccattccctatgatatcaaggtctggcgggatctcagcggcggggccggggaggccgggctggacgagatggcgggccgggcctgccggttcctcaaggagctgaccgcgtaa

SEQ ID NO: 11 - DNA, 885 bp, Artificial Sequence
  Polynucleotide coding D-allulose 3-epimerase variant W29K/W209L/G216S/M234I
atgaacccgattggaatgcactacggcttctggagccacaactgggacgagattgcatacatacccctgatggagaagctggccaaactgggctttgacatctgcgaggtggcctccgccgagtggggctattacgacgacgccaggctgcgggagctgaaggcctgcgccgatcacaacggcctgggcatcacctattccatcggcctggaggccaaatacgacctggccagcgacgatccggcggtgcgggagaacggcatccgccatgtcacccgcatcctggagagcatgcccaaggtgggggcggccatcctcaacggcgtgtcctacgccgggtggcaggccctgcccgaccacggaatcaccctggacgagaagcgccgcaaggaggagcttgccctggagtccatgtcccggctcatgaaggtggcggaggactgcggcgtgctctactgctgcgaggtggtcaaccgcttcgagcagtacctgctcaacaccgccaaagagggcgtggagtttgtcaagcgcctgggcagtcccaacgcccgggtgctgctggataccttccacatgaacatcgaggaggacagcatggtggacgccattctggaggcgggccccctgctggggcatttccacgtgagcgagaacaaccgccgccccgccggctccaccaaccgcctgccctggaaggacattgccgccgccctcaagcaggtgaactaccagggggccattgtgatggagcccttcgtgctcatggggggtaccattccctatgatatcaaggtctggcgggatctcagcggcggggccggggaggccgggctggacgagatggcgggccgggcctgccggttcctcaaggagctgaccgcgtaa

SEQ ID NO: 12 - DNA, 885 bp, Artificial Sequence
  Polynucleotide coding D-allulose 3-epimerase variant W29K/G216S/M234I/Q240D
atgaacccgattggaatgcactacggcttctggagccacaactgggacgagattgcatacatacccctgatggagaagctggccaaactgggctttgacatctgcgaggtggcctccgccgagtggggctattacgacgacgccaggctgcgggagctgaaggcctgcgccgatcacaacggcctgggcatcacctattccatcggcctggaggccaaatacgacctggccagcgacgatccggcggtgcgggagaacggcatccgccatgtcacccgcatcctggagagcatgcccaaggtgggggcggccatcctcaacggcgtgtcctacgccgggtggcaggccctgcccgaccacggaatcaccctggacgagaagcgccgcaaggaggagcttgccctggagtccatgtcccggctcatgaaggtggcggaggactgcggcgtgctctactgctgcgaggtggtcaaccgcttcgagcagtacctgctcaacaccgccaaagagggcgtggagtttgtcaagcgcctgggcagtcccaacgcccgggtgctgctggataccttccacatgaacatcgaggaggacagcatggtggacgccattctggaggcgggcccctggctggggcatttccacgtgagcgagaacaaccgccgccccgccggctccaccaaccgcctgccctggaaggacattgccgccgccctcaaggatgtgaactaccagggggccattgtgatggagcccttcgtgctcatggggggtaccattccctatgatatcaaggtctggcgggatctcagcggcggggccggggaggccgggctggacgagatggcgggccgggcctgccggttcctcaaggagctgaccgcgtaa